European Patent Specification EP 3 645 560 B1, published December 20, 2023. Title: Treatment of haematological malignancies. Applicant: Academisch Ziekenhuis Leiden (handelend onder de naam Leids Universitair Medisch Centrum/ h.o.d.n. LUMC). The sequence listing filed with the application follows.

SEQUENCE LISTING (31 sequences)

SEQ ID NO: 1 - protein, 9 aa, Homo sapiens
CLAVEEVSL

SEQ ID NO: 2 - protein, 10 aa, Homo sapiens
CAVTGARLMF

SEQ ID NO: 3 - DNA, 30 bp, Homo sapiens
tgtgccgttacgggggccagactcatgttt

SEQ ID NO: 4 - DNA, 30 bp, Artificial Sequence
  optimised nucleic acid sequence encoding CDR3 (TCR alpha chain)
tgcgcagtgacaggagcaaggctgatgttc

SEQ ID NO: 5 - protein, 13 aa, Homo sapiens
CASSPGGLSNEQF

SEQ ID NO: 6 - DNA, 39 bp, Homo sapiens
tgcgccagcagccctggcggcttgtccaatgagcagttc

SEQ ID NO: 7 - DNA, 39 bp, Artificial Sequence
  optimised nucleic acid sequence encoding CDR3 (TCR beta chain)
tgcgcaagctccccaggaggcctgtccaacgagcagttc

SEQ ID NO: 8 - protein, 129 aa, Homo sapiens
MKSLRVLLVILWLQLSWVWSQQKEVEQNSGPLSVPEGAIASLNCTYSDRGSQSFFWYRQYSGKSPELIMFIYSNGDKEDGRFTAQLNKASQYVSLLIRDSQPSDSATYLCAVTGARLMFGDGTQLVVKP

SEQ ID NO: 9 - DNA, 387 bp, Homo sapiens
atgaaatccttgagagttttactagtgatcctgtggcttcagttgagctgggtttggagccaacagaaggaggtggagcagaattctggacccctcagtgttccagagggagccattgcctctctcaactgcacttacagtgaccgaggttcccagtccttcttctggtacagacaatattctgggaaaagccctgagttgataatgttcatatactccaatggtgacaaagaagatggaaggtttacagcacagctcaataaagccagccagtatgtttctctgctcatcagagactcccagcccagtgattcagccacctacctctgtgccgttacgggggccagactcatgtttggagatggaactcagctggtggtgaagccc

SEQ ID NO: 10 - DNA, 387 bp, Artificial Sequence
  optimised nucleic acid sequence encoding alpha chain variable region
atgaaatccttgagagttttactagtgatcctgtggcttcaattgagctgggtgtggtcccagcagaaggaggtggagcagaactctggaccactgagcgtgccagagggagccatcgccagcctgaattgcacctactccgaccggggcagccagtccttcttttggtacagacagtattccggcaagtctcccgagctgatcatgttcatctattctaacggcgacaaggaggatggcaggtttacagcccagctgaataaggcctcccagtacgtgtctctgctgatccgcgactcccagccttctgatagcgccacctacctgtgcgcagtgacaggagcaaggctgatgttcggcgacggaacccagctggtggtgaagcca

SEQ ID NO: 11 - protein, 132 aa, Homo sapiens
MGSRLLCWVLLCLLGAGPVKAGVTQTPRYLIKTRGQQVTLSCSPISGHRSVSWYQQTPGQGLQFLFEYFSETQRNKGNFPGRFSGRQFSNSRSEMNVSTLELGDSALYLCASSPGGLSNEQFFGPGTRLTVL

SEQ ID NO: 12 - DNA, 396 bp, Homo sapiens
atgggctccaggctgctctgttgggtgctgctttgtctcctgggagcaggcccagtaaaggctggagtcactcaaactccaagatatctgatcaaaacgagaggacagcaagtgacactgagctgctcccctatctctgggcataggagtgtatcctggtaccaacagaccccaggacagggccttcagttcctctttgaatacttcagtgagacacagagaaacaaaggaaacttccctggtcgattctcagggcgccagttctctaactctcgctctgagatgaatgtgagcaccttggagctgggggactcggccctttatctttgcgccagcagccctggcggcttgtccaatgagcagttcttcgggccagggacacggctcaccgtgcta

SEQ ID NO: 13 - DNA, 396 bp, Artificial Sequence
  optimised nucleic acid sequence encoding beta chain variable region
atgggctccaggctgctgtgctgggtgctgctgtgcctgctgggagcaggaccagtgaaggcaggcgtgacccagacacctaggtacctgatcaagacccgcggccagcaggtgacactgtcttgcagccctatctctggccaccgctccgtgtcttggtaccagcagaccccaggacagggcctgcagttcctgtttgagtatttctctgagacacagcggaacaagggcaatttccccggccggtttagcggcagacagtttagcaactccagatctgagatgaatgtgagcaccctggagctgggcgactccgccctgtacctgtgcgcaagctccccaggaggcctgtccaacgagcagttctttggaccaggaaccaggctgacagtgctg

SEQ ID NO: 14 - protein, 7 aa, Homo sapiens
SDRGSQS

SEQ ID NO: 15 - protein, 7 aa, Homo sapiens
FIYSNGD

SEQ ID NO: 16 - protein, 5 aa, Homo sapiens
SGHRS

SEQ ID NO: 17 - protein, 13 aa, Homo sapiens
EYFSETQRNKGNF

SEQ ID NO: 18 - DNA, 21 bp, Homo sapiens
agtgaccgaggttcccagtcc

SEQ ID NO: 19 - DNA, 21 bp, Artificial Sequence
  optimised nucleic acid sequence encoding CDR1 (TCR alpha chain)
tccgaccggggcagccagtcc

SEQ ID NO: 20 - DNA, 21 bp, Homo sapiens
ttcatatactccaatggtgac

SEQ ID NO: 21 - DNA, 21 bp, Artificial Sequence
  optimised nucleic acid sequence encoding CDR2 (TCR alpha chain)
ttcatctattctaacggcgac

SEQ ID NO: 22 - DNA, 15 bp, Homo sapiens
tctgggcataggagt

SEQ ID NO: 23 - DNA, 15 bp, Artificial Sequence
  optimised nucleic acid sequence encoding CDR1 (TCR beta chain)
tctggccaccgctcc

SEQ ID NO: 24 - DNA, 39 bp, Homo sapiens
gaatacttcagtgagacacagagaaacaaaggaaacttc

SEQ ID NO: 25 - DNA, 39 bp, Artificial Sequence
  optimised nucleic acid sequence encoding CDR2 (TCR beta chain)
gagtatttctctgagacacagcggaacaagggcaatttc

SEQ ID NO: 26 - protein, 9 aa, Homo sapiens
AVEEVSLRK

SEQ ID NO: 27 - protein, 11 aa, Homo sapiens
CLAVEEVSLRK

SEQ ID NO: 28 - protein, 8 aa, Homo sapiens
VEEVSLRK

SEQ ID NO: 29 - protein, 8 aa, Homo sapiens
AVEEVSLR

SEQ ID NO: 30 - protein, 21 aa, Homo sapiens
MTDQEAIQDLCLAVEEVSLRK

SEQ ID NO: 31 - protein, 9 aa, Cytomegalovirus
NLVPMVATV